European Patent Application EP 4 190 362 A1, published June 7, 2023. Title: A therapeutic agent for EGFR mutation positive lung cancer comprising REIC/Dkk-3 gene. Applicant: National University Corporation Okayama University Momotaro-Gene Inc. The sequence listing filed with the application follows.

SEQUENCE LISTING (7 sequences)

SEQ ID NO: 1 - DNA, 1053 bp, Homo sapiens
  CDS (1)..(1053)
atgcagcggcttggggccaccctgctgtgcctgctactggcggcggcggtccccacggcccccgcgcccgctccgacggcgacctcggctccagtcaagcccggcccggctctcagctacccgcaggaggaggccaccctcaatgagatgttccgcgaggttgaggaactggtggaggacacgcagcacaaattgcgcagcgcggtggaagagatggaggcagaagaagctgctgctaaagcatcatcagaagtgaacctggcaaacttacctcccagctatcacaatgagaccaacacagacacgaaggttggaaataataccatccatgtgcaccgagaaattcacaagataaccaacaaccaggctcgacaaatggtcttttcagagacagttatcacatctgtgggagacgaagaaggcagaaggagccacgagtgcatcatcgacgaggactgtgggcccagcatgtactgccagtttgccagcttccagtacacctgccagccatgccggggccagaggatgctctgcacccgggacagtgagtgctgtggagaccagctgtgtgtctggggtcactgcaccaaaatggccaccaggggcagcaatgggaccatctgtgacaaccagagggactgccagccggggctgtgctgtgccttccagagaggcctgctgttccctgtgtgcatacccctgcccgtggagggcgagctttgccatgaccccgccagccggcttctggacctcatcacctgggagctagagcctgatggagccttggaccgatgcccttgtgccagtggcctcctctgccagccccacagccacagcctggtgtatgtgtgcaagccgaccttcgtggggagccgtgaccaagatggggagatcctgctgcccagagaggtccccgatgagtatgaagttggcagcttcatggaggaggtgcgccaggagctggaggacctggagaggagcctgactgaagagatggcgctgggggagcctgcggctgccgccgctgcactgctgggaggggaagagatttag

SEQ ID NO: 2 - protein, 350 aa, Homo sapiens [sequence omitted]

SEQ ID NO: 3 - DNA, 117 bp, Homo sapiens
atgcagcggcttggggccaccctgctgtgcctgctactggcggcggcggtccccacggcccccgcgcccgctccgacggcgacctcggctccagtcaagcccggcccggctctcagc

SEQ ID NO: 4 - DNA, 234 bp, Homo sapiens
atgcagcggcttggggccaccctgctgtgcctgctactggcggcggcggtccccacggcccccgcgcccgctccgacggcgacctcggctccagtcaagcccggcccggctctcagctacccgcaggaggaggccaccctcaatgagatgttccgcgaggttgaggaactggtggaggacacgcagcacaaattgcgcagcgcggtggaagagatggaggcagaagaagctgct

SEQ ID NO: 5 - DNA, 262 bp, Artificial
  Synthetic
tgactgactgacgtttaaacccgctgatcagcctcgactgtgccttctagttgccagccatctgttgtttgcccctcccccgtgccttccttgaccctggaaggtgccactcccactgtcctttcctaataaaatgaggaaattgcatcgcattgtctgagtaggtgtcattctattctggggggtggggtggggcaggacagcaagggggaggattgggaagacaatagcaggcatgctggggatgcggtgggctctatgg

SEQ ID NO: 6 - DNA, 2355 bp, Artificial
  Synthetic
tctagagcaccatgcagcggcttggggccaccctgctgtgcctgctgctggcggcggcggtccccacggcccccgcgcccgctccgacggcgacctcggctccagtcaagcccggcccggctctcagctacccgcaggaggaggccaccctcaatgagatgttccgcgaggttgaggaactgatggaggacacgcagcacaaattgcgcagcgcggtggaagagatggaggcagaagaagctgctgctaaagcatcatcagaagtgaacctggcaaacttacctcccagctatcacaatgagaccaacacagacacgaaggttggaaataataccatccatgtgcaccgagaaattcacaagataaccaacaaccagactggacaaatggtcttttcagagacagttatcacatctgtgggagacgaagaaggcagaaggagccacgagtgcatcatcgacgaggactgtgggcccagcatgtactgccagtttgccagcttccagtacacctgccagccatgccggggccagaggatgctctgcacccgggacagtgagtgctgtggagaccagctgtgtgtctggggtcactgcaccaaaatggccaccaggggcagcaatgggaccatctgtgacaaccagagggactgccagccggggctgtgctgtgccttccagagaggcctgctgttccctgtgtgcacacccctgcccgtggagggcgagctttgccatgaccccgccagccggcttctggacctcatcacctgggagctagagcctgatggagccttggaccgatgcccttgtgccagtggcctcctctgccagccccacagccacagcctggtgtatgtgtgcaagccgaccttcgtggggagccgtgaccaagatggggagatcctgctgcccagagaggtccccgatgagtatgaagttggcagcttcatggaggaggtgcgccaggagctggaggacctggagaggagcctgactgaagagatggcgctgggggagcctgcggctgccgccgctgcactgctgggaggggaagagatttagggggtaccccggctagatgactaacgtttaaacccgctgatcagcctcgactgtgccttctagttgccagccatctgttgtttgcccctcccccgtgccttccttgaccctggaaggtgccactcccactgtcctttcctaataaaatgaggaaattgcatcgcattgtctgagtaggtgtcattctattctggggggtggggtggggcaggacagcaagggggaggattgggaagacaatagcaggcatgctggggatgcggtgggctctatggcggagtactgtcctccgcttcccacgtggcggagggactggggacccgggcacccgtcctgccccttcaccttccagctccgcctcctccgcgcggaccccgccccgtcccgacccctcccgggtccccggcccagccccctccgggccctcccagcccctccccttcctttccgcggccccgccctctcctcgcggcgcgagttttggaaagtccccaggctccccagcaggcagaagtatccaaagcatccatctcaattagtcagcaaccaggtgtggaaagtccccaggctccccagcaggcagaagtatccaaagcatccatctcaattagtcagcaaccatagtcccgcccctaactccgcccatcccgcccctaactccgcccagttccgcccattctccgccccatggctgactaattttttttatttatgcagaggccgaggccgcctctgcctctgagctattccagaagtagtgaggaggcttttttggaggccaaggcttttgcaaaaagctccgttacataacttacggtaaatggcccgcctggctgaccgcccaacgacccccgcccattgacgtcaataatgacgtatgttcccatagtaacgccaatagggactttccattgacgtcaatgggtggagtatttacggtaaactgcccacttggcagtacatcaagtgtatcatatgccaagtacgccccctattgacgtcaatgacggtaaatggcccgcctggcattatgcccagtacatgaccttatgggactttcctacttggcagtacatctacgtattagtcatcgctattaccatggtgatgcggttttggcagtacatcaatgggcgtggatagcggtttgactcacggggatttccaagtctccaccccattgacgtcaatgggagtttgttttggcaccaaaatcaacgggactttccaaaatgtcgtaacaactccgccccattgacgcaaatgggcggtaggcgtgttgccggaattc

SEQ ID NO: 7 - DNA, 1285 bp, Artificial
  Synthetic
gtttaaacccgctgatcagcctcgactgtgccttctagttgccagccatctgttgtttgcccctcccccgtgccttccttgaccctggaaggtgccactcccactgtcctttcctaataaaatgaggaaattgcatcgcattgtctgagtaggtgtcattctattctggggggtggggtggggcaggacagcaagggggaggattgggaagacaatagcaggcatgctggggatgcggtgggctctatggcggagtactgtcctccgcttcccacgtggcggagggactggtcctccgcttcccacgtggcggagggactggggacccgggcacccgtcctgccccttcaccttccagctccgcctcctccgcgcggaccccgccccgtcccgacccctcccgggtccccggcccagccccctccgggccctcccagcccctccccttcctttccgcggccccgccctctcctcgcggcgcgagttttggaaagtccccaggctccccagcaggcagaagtatccaaagcatccatctcaattagtcagcaaccaggtgtggaaagtccccaggctccccagcaggcagaagtatccaaagcatccatctcaattagtcagcaaccatagtcccgcccctaactccgcccatcccgcccctaactccgcccagttccgcccattctccgccccatggctgactaattttttttatttatgcagaggccgaggccgcctctgcctctgagctattccagaagtagtgaggaggcttttttggaggccaaggcttttgcaaaaagctccgttacataacttacggtaaatggcccgcctggctgaccgcccaacgacccccgcccattgacgtcaataatgacgtatgttcccatagtaacgccaatagggactttccattgacgtcaatgggtggagtatttacggtaaactgcccacttggcagtacatcaagtgtatcatatgccaagtacgccccctattgacgtcaatgacggtaaatggcccgcctggcattatgcccagtacatgaccttatgggactttcctacttggcagtacatctacgtattagtcatcgctattaccatggtgatgcggttttggcagtacatcaatgggcgtggatagcggtttgactcacggggatttccaagtctccaccccattgacgtcaatgggagtttgttttggcaccaaaatcaacgggactttccaaaatgtcgtaacaactccgccccattgacgcaaatgggcggtaggcgtg